European Patent Application EP 4 715 043 A1, published March 25, 2026. Title: Method for producing neural crest cell. Applicant: Kyoto University. The sequence listing filed with the application follows.

SEQUENCE LISTING (20 sequences)

SEQ ID NO: 1 - DNA, 25 bp, synthetic construct
  source 1..25: mol_type = other DNA
  misc_feature 1..25: note = PCR Primer
gcatcaccaaacaaaaactcctttg

SEQ ID NO: 2 - DNA, 25 bp, synthetic construct
  source 1..25: mol_type = other DNA
  misc_feature 1..25: note = PCR Primer
tgggtcagggaatcactaaacagaa

SEQ ID NO: 3 - DNA, 25 bp, synthetic construct
  source 1..25: mol_type = other DNA
  misc_feature 1..25: note = PCR Primer
accaactaacgcctaaacctcggta

SEQ ID NO: 4 - DNA, 25 bp, synthetic construct
  source 1..25: mol_type = other DNA
  misc_feature 1..25: note = PCR Primer
gcagatttttggagcaattctttcc

SEQ ID NO: 5 - DNA, 20 bp, synthetic construct
  source 1..20: mol_type = other DNA
  misc_feature 1..20: note = PCR Primer
ttcaccagtacgctctgtgc

SEQ ID NO: 6 - DNA, 20 bp, synthetic construct
  source 1..20: mol_type = other DNA
  misc_feature 1..20: note = PCR Primer
ttttccagtagacggccaag

SEQ ID NO: 7 - DNA, 21 bp, synthetic construct
  source 1..21: mol_type = other DNA
  misc_feature 1..21: note = PCR Primer
ggaagcgctttgcacaaacta

SEQ ID NO: 8 - DNA, 20 bp, synthetic construct
  source 1..20: mol_type = other DNA
  misc_feature 1..20: note = PCR Primer
ttcaccattctcacctcggg

SEQ ID NO: 9 - DNA, 21 bp, synthetic construct
  source 1..21: mol_type = other DNA
  misc_feature 1..21: note = PCR Primer
tgatgcttttgtgcgagaaga

SEQ ID NO: 10 - DNA, 21 bp, synthetic construct
  source 1..21: mol_type = other DNA
  misc_feature 1..21: note = PCR Primer
agggaagcgtttttattggct

SEQ ID NO: 11 - DNA, 22 bp, synthetic construct
  source 1..22: mol_type = other DNA
  misc_feature 1..22: note = PCR Primer
gccaggtacatcgacttcctct

SEQ ID NO: 12 - DNA, 22 bp, synthetic construct
  source 1..22: mol_type = other DNA
  misc_feature 1..22: note = PCR Primer
tccatcctccagaccgagaagg

SEQ ID NO: 13 - DNA, 20 bp, synthetic construct
  source 1..20: mol_type = other DNA
  misc_feature 1..20: note = PCR Primer
acagtgctgctccttctggt

SEQ ID NO: 14 - DNA, 20 bp, synthetic construct
  source 1..20: mol_type = other DNA
  misc_feature 1..20: note = PCR Primer
atgtgagacctgggaattgg

SEQ ID NO: 15 - DNA, 20 bp, synthetic construct
  source 1..20: mol_type = other DNA
  misc_feature 1..20: note = PCR Primer
caagcacaatttgctcagga

SEQ ID NO: 16 - DNA, 20 bp, synthetic construct
  source 1..20: mol_type = other DNA
  misc_feature 1..20: note = PCR Primer
ggcacgtaggcagaataagc

SEQ ID NO: 17 - DNA, 23 bp, synthetic construct
  source 1..23: mol_type = other DNA
  misc_feature 1..23: note = PCR Primer
gaggagaaagtggaggtctggtt

SEQ ID NO: 18 - DNA, 21 bp, synthetic construct
  source 1..21: mol_type = other DNA
  misc_feature 1..21: note = PCR Primer
ctctgatgaggaccgcttctg

SEQ ID NO: 19 - DNA, 20 bp, synthetic construct
  source 1..20: mol_type = other DNA
  misc_feature 1..20: note = PCR Primer
agcgcaagttccgtcagaaa

SEQ ID NO: 20 - DNA, 20 bp, synthetic construct
  source 1..20: mol_type = other DNA
  misc_feature 1..20: note = PCR Primer
acctgggtctctgtgaggtt